European Patent Application EP 4 790 066 A1, published August 12, 2026. Title: GLP-1R/GIPR/GCGR三重激动剂类似物及其用途. Applicant: 深圳湾实验室. Application CN. The sequence listing filed with the application follows.

SEQUENCE LISTING (94 sequences)

SEQ ID NO: 1 - protein, 39 aa, synthetic construct
  VARIANT 2: note = X=Aib
YXQGTFTSDYSKYCDKRAAQCFVQWLLAGGPSSGAPPPS

SEQ ID NO: 2 - protein, 39 aa, synthetic construct
  VARIANT 2: note = X=Aib
YXQGTFTSDYSKYCDEKRAKCFVQWLLDHHPSSGQPPPS

SEQ ID NO: 3 - protein, 39 aa, synthetic construct
  VARIANT 2: note = X=Aib
YXQGTFTSDCSKYCDERAAQDFVQWLLAGGPSSGAPPPS

SEQ ID NO: 4 - protein, 39 aa, synthetic construct
  VARIANT 2: note = X=Aib
YXQGTFTSDCSKYLDECAAQDFVQWLLAGGPSSGAPPPS

SEQ ID NO: 5 - protein, 39 aa, synthetic construct
  VARIANT 2: note = X=Aib
YXQGTFTSDCSKYLDERAAQCFVQWLLAGGPSSGAPPPS

SEQ ID NO: 6 - protein, 39 aa, synthetic construct
  VARIANT 2: note = X=Aib
HXHGTFTSDYSIYCEKKYAQCFVQWLLAGGPSSGAPPPS

SEQ ID NO: 7 - protein, 39 aa, synthetic construct
  VARIANT 2: note = X=Aib
HXHGTFTSDYSIYCEKRYAQCFVQWLLAGGPSSGAPPPS

SEQ ID NO: 8 - protein, 39 aa, synthetic construct
  VARIANT 2: note = X=Aib
  VARIANT 20: note = X=Aib
HXHGTFTSDYSIYCEKRYAXCFVQWLLEGGPSSGAPPPS

SEQ ID NO: 9 - protein, 39 aa, synthetic construct
  VARIANT 2: note = X=Aib
YXQGTFTSDYSKYLDKCAAQDFVCWLLAGGPSSGAPPPS

SEQ ID NO: 10 - protein, 39 aa, synthetic construct
  VARIANT 2: note = X=Aib
HXHGTFTSDYSKYLDKCYAQDFVCWLLEGGPSSGAPPPS

SEQ ID NO: 11 - protein, 39 aa, synthetic construct
  VARIANT 2: note = X=Aib
YXQGTFTSDYSILLDKCAQHAFICYLLEGGPSSGAPPPS

SEQ ID NO: 12 - protein, 39 aa, synthetic construct
  VARIANT 2: note = X=Aib
  VARIANT 20: note = X=Aib
YXQGTFTSDYSILLDKCAQXAFICYLLEGGPSSGAPPPS

SEQ ID NO: 13 - protein, 39 aa, synthetic construct
  VARIANT 2: note = X=Aib
HXHGTFTSDYSRALEKCAARLFICWLLEGGPSSGAPPPS

SEQ ID NO: 14 - protein, 39 aa, synthetic construct
  VARIANT 2: note = X=Aib
  VARIANT 16: note = X=K(Ac)
  VARIANT 20: note = X=Aib
HXHGTFTSDYSKYLEXKYAXCFVQWLLCGGPSSGAPPPS

SEQ ID NO: 15 - protein, 39 aa, synthetic construct
  VARIANT 2: note = X=Aib
  VARIANT 13: note = X=aMeL
  VARIANT 17: note = X=K(Ac)
  VARIANT 20: note = X=Aib
YXQGTFTSDYSIXLDKXAQXCFIEYLLCGGPSSGAPPPS

SEQ ID NO: 16 - protein, 39 aa, synthetic construct
  VARIANT 2: note = X=Aib
  VARIANT 14: note = X=K(Ac)
  VARIANT 20: note = X=Aib
  VARIANT 34: note = X=Aib
HXHGTFTSDLSKLXEEQRQXCFIEWLKCGGPPSXKPPPK

SEQ ID NO: 17 - protein, 39 aa, synthetic construct
  VARIANT 2: note = X=Aib
  VARIANT 14: note = X=K(Ac)
HXQGTFTSDLSKQXDEQRAKCFIEWLICGGPSSGAPPPS

SEQ ID NO: 18 - protein, 39 aa, synthetic construct
  VARIANT 2: note = X=Aib
  VARIANT 13: note = X=aMeL
  VARIANT 17: note = X=K(Ac)
  VARIANT 20: note = X=Aib
HXQGTFTSDYSIXLDKXAQXCFIEYLLCGGPSSGAPPPS

SEQ ID NO: 19 - protein, 39 aa, synthetic construct
  VARIANT 1: note = X=3-iodo-Y
  VARIANT 2: note = X=Aib
  VARIANT 13: note = X=aMeL
  VARIANT 17: note = X=K(Ac)
  VARIANT 20: note = X=Aib
XXQGTFTSDYSIXLDKXAQXCFIEYLLCGGPSSGAPPPS

SEQ ID NO: 20 - protein, 39 aa, synthetic construct; identical to SEQ ID NO: 19
  VARIANT 1: note = X=4-Pal
  VARIANT 2: note = X=Aib
  VARIANT 13: note = X=aMeL
  VARIANT 17: note = X=K(Ac)
  VARIANT 20: note = X=Aib

SEQ ID NO: 21 - protein, 39 aa, synthetic construct; identical to SEQ ID NO: 19
  VARIANT 1: note = X=4-amino-F
  VARIANT 2: note = X=Aib
  VARIANT 13: note = X=aMeL
  VARIANT 17: note = X=K(Ac)
  VARIANT 20: note = X=Aib

SEQ ID NO: 22 - protein, 39 aa, synthetic construct; identical to SEQ ID NO: 15
  VARIANT 2: note = X=s
  VARIANT 13: note = X=aMeL
  VARIANT 17: note = X=K(Ac)
  VARIANT 20: note = X=Aib

SEQ ID NO: 23 - protein, 39 aa, synthetic construct
  VARIANT 2: note = X=Aib
  VARIANT 6: note = X=aMeF
  VARIANT 13: note = X=aMeL
  VARIANT 17: note = X=K(Ac)
  VARIANT 20: note = X=Aib
YXQGTXTSDYSIXLDKXAQXCFIEYLLCGGPSSGAPPPS

SEQ ID NO: 24 - protein, 39 aa, synthetic construct
  VARIANT 2: note = X=Aib
  VARIANT 8: note = X=HoS
  VARIANT 13: note = X=aMeL
  VARIANT 17: note = X=K(Ac)
  VARIANT 20: note = X=Aib
YXQGTFTXDYSIXLDKXAQXCFIEYLLCGGPSSGAPPPS

SEQ ID NO: 25 - protein, 39 aa, synthetic construct
  VARIANT 2: note = X=Aib
  VARIANT 13: note = X=aMeL
  VARIANT 14: note = X=HoL
  VARIANT 17: note = X=K(Ac)
  VARIANT 20: note = X=Aib
YXQGTFTSDYSIXXDKXAQXCFIEYLLCGGPSSGAPPPS

SEQ ID NO: 26 - protein, 39 aa, synthetic construct; identical to SEQ ID NO: 25
  VARIANT 2: note = X=Aib
  VARIANT 13: note = X=aMeL
  VARIANT 14: note = X=Npg
  VARIANT 17: note = X=K(Ac)
  VARIANT 20: note = X=Aib

SEQ ID NO: 27 - protein, 39 aa, synthetic construct; identical to SEQ ID NO: 25
  VARIANT 2: note = X=Aib
  VARIANT 13: note = X=aMeL
  VARIANT 14: note = X=Tle
  VARIANT 20: note = X=Aib

SEQ ID NO: 28 - protein, 39 aa, synthetic construct
  VARIANT 2: note = X=Aib
  VARIANT 13: note = X=aMeL
  VARIANT 17: note = X=K(Ac)
  VARIANT 20: note = X=Aib
YXQGTFTSDYSIXLDKXAQXCFIEWLLCGGPSSGAPPPS

SEQ ID NO: 29 - protein, 39 aa, synthetic construct
  VARIANT 2: note = X=Aib
  VARIANT 17: note = X=K(Ac)
  VARIANT 20: note = X=Aib
YXQGTFTSDYSILLDKXAQXCFIEWLLCGGPSSGAPPPS

SEQ ID NO: 30 - protein, 39 aa, synthetic construct
  VARIANT 2: note = X=Aib
  VARIANT 13: note = X=aMeL
  VARIANT 20: note = X=Aib
YXQGTFTSDYSIXLDKQAQXCFIEYLLCGGPSSGAPPPS

SEQ ID NO: 31 - protein, 39 aa, synthetic construct; identical to SEQ ID NO: 15
  VARIANT 2: note = X=Aib
  VARIANT 13: note = X=aMeL
  VARIANT 17: note = X=K(Ac)
  VARIANT 20: note = X=a

SEQ ID NO: 32 - protein, 39 aa, synthetic construct
  VARIANT 2: note = X=Aib
  VARIANT 13: note = X=aMeL
  VARIANT 17: note = X=K(Ac)
YXQGTFTSDYSIXLDKXAQHCFIEYLLCGGPSSGAPPPS

SEQ ID NO: 33 - protein, 39 aa, synthetic construct
  VARIANT 2: note = X=Aib
  VARIANT 13: note = X=aMeL
  VARIANT 17: note = X=K(Ac)
YXQGTFTSDYSIXLDKXAQQCFIEYLLCGGPSSGAPPPS

SEQ ID NO: 34 - protein, 39 aa, synthetic construct
  VARIANT 2: note = X=Aib
  VARIANT 13: note = X=aMeL
  VARIANT 17: note = X=K(Ac)
  VARIANT 19: note = X=Aib
YXQGTFTSDYSIXLDKXAXQCFIEYLLCGGPSSGAPPPS

SEQ ID NO: 35 - protein, 39 aa, synthetic construct
  VARIANT 2: note = X=Aib
  VARIANT 13: note = X=aMeL
  VARIANT 20: note = X=Aib
YXQGTFTSDYSIXLDKRAQXCFIEYLLCGGPSSGAPPPS

SEQ ID NO: 36 - protein, 39 aa, synthetic construct
  VARIANT 2: note = X=Aib
  VARIANT 13: note = X=aMeL
  VARIANT 17: note = X=K(Ac)
  VARIANT 20: note = X=Aib
YXQGTFTSDYSIXLEKXAQXCFIEYLLCGGPSSGAPPPS

SEQ ID NO: 37 - protein, 39 aa, synthetic construct
  VARIANT 2: note = X=Aib
  VARIANT 13: note = X=aMeL
  VARIANT 15: note = X=Aad
YXQGTFTSDYSIXLXKXAQXCFIEYLLCGGPSSGAPPPS

SEQ ID NO: 38 - protein, 39 aa, synthetic construct
  VARIANT 2: note = X=Aib
  VARIANT 10: note = X=4-Pal
  VARIANT 13: note = X=aMeL
  VARIANT 17: note = X=K(Ac)
  VARIANT 20: note = X=Aib
YXQGTFTSDXSIXLDKXAQXCFIEYLLCGGPSSGAPPPS

SEQ ID NO: 39 - protein, 39 aa, synthetic construct; identical to SEQ ID NO: 24
  VARIANT 2: note = X=Aib
  VARIANT 8: note = X=aMeS
  VARIANT 13: note = X=aMeL
  VARIANT 17: note = X=K(Ac)
  VARIANT 20: note = X=Aib

SEQ ID NO: 40 - protein, 39 aa, synthetic construct; identical to SEQ ID NO: 23
  VARIANT 2: note = X=Aib
  VARIANT 6: note = X=F(2-F)
  VARIANT 13: note = X=aMeL
  VARIANT 17: note = X=K(Ac)
  VARIANT 20: note = X=Aib

SEQ ID NO: 41 - protein, 39 aa, synthetic construct
  VARIANT 2: note = X=Aib
  VARIANT 3: note = X=Dab(Ac)
  VARIANT 13: note = X=aMeL
  VARIANT 17: note = X=K(Ac)
  VARIANT 20: note = X=Aib
YXXGTFTSDYSIXLDKXAQXCFIEYLLCGGPSSGAPPPS

SEQ ID NO: 42 - protein, 39 aa, synthetic construct
  VARIANT 2: note = X=Aib
  VARIANT 13: note = X=aMeL
  VARIANT 17: note = X=K(Ac)
  VARIANT 20: note = X=Aib
YXHGTFTSDYSIXLDKXAQXCFIEYLLCGGPSSGAPPPS

SEQ ID NO: 43 - protein, 39 aa, synthetic construct; identical to SEQ ID NO: 15
  VARIANT 2: note = X=Ac4c
  VARIANT 13: note = X=aMeL
  VARIANT 17: note = K(Ac)
  VARIANT 20: note = X=Aib

SEQ ID NO: 44 - protein, 39 aa, synthetic construct
  VARIANT 2: note = X=Aib
  VARIANT 21: note = X=Aib
YXQGTFTSDYSILLDKCAQHXFIEYLLCGGPSSGAPPPS

SEQ ID NO: 45 - protein, 39 aa, synthetic construct
  VARIANT 2: note = X=Aib
  VARIANT 17: note = X=HoC
  VARIANT 21: note = X=Aib
  VARIANT 28: note = X=HoC
YXQGTFTSDYSILLDKXAQHXFIEYLLXGGPSSGAPPPS

SEQ ID NO: 46 - protein, 39 aa, synthetic construct
  VARIANT 2: note = X=Aib
  VARIANT 6: note = X=F(2-F)
YXQGTXTSDYSILLDKCAQQAFICYLLAGGPSSGAPPPS

SEQ ID NO: 47 - protein, 39 aa, synthetic construct
  VARIANT 2: note = X=Aib
  VARIANT 6: note = X=F(2-F)
YXQGTXTSDYSILLDKQAQQCFIEYLLCGGPSSGAPPPS

SEQ ID NO: 48 - protein, 39 aa, synthetic construct
  VARIANT 2: note = X=Aib
  VARIANT 6: note = X=F(2-F)
  VARIANT 13: note = X=Aib
  VARIANT 17: note = X=K(Ac)
YXQGTXTSDYSIXLDKXAQQCFIEYLLCGGPSSGAPPPS

SEQ ID NO: 49 - protein, 39 aa, synthetic construct
  VARIANT 2: note = X=Aib
  VARIANT 6: note = X=F(2-F)
YXQGTXTSDYSILCDKQAQQCFIEYLLAGGPSSGAPPPS

SEQ ID NO: 50 - protein, 39 aa, synthetic construct
  VARIANT 2: note = X=Aib
  VARIANT 6: note = X=F(2-F)
  VARIANT 16: note = X=aMeK
  VARIANT 17: note = X=K(Ac)
YXQGTXTSDYSILLDXXAQQCFIEYLLCGGPSSGAPPPS

SEQ ID NO: 51 - protein, 39 aa, synthetic construct
  VARIANT 2: note = X=Aib
  VARIANT 6: note = X=F(2-F)
  VARIANT 16: note = X=aMeK
  VARIANT 17: note = X=K(Ac)
  VARIANT 20: note = X=Aib
YXQGTXTSDYSILLDXXAQXCFIEYLICGGPSSGAPPPS

SEQ ID NO: 52 - protein, 39 aa, synthetic construct; identical to SEQ ID NO: 23
  VARIANT 2: note = X=Aib
  VARIANT 6: note = X=F(2-F)
  VARIANT 13: note = X=Iva
  VARIANT 17: note = X=K(Ac)
  VARIANT 20: note = X=Aib

SEQ ID NO: 53 - protein, 39 aa, synthetic construct; identical to SEQ ID NO: 23
  VARIANT 2: note = X=Aib
  VARIANT 6: note = X=F(2-F)
  VARIANT 13: note = X=Iva
  VARIANT 17: note = X=K(Ac)
  VARIANT 20: note = X=Aib

SEQ ID NO: 54 - protein, 39 aa, synthetic construct; identical to SEQ ID NO: 23
  VARIANT 2: note = X=Aib
  VARIANT 6: note = X=F(2-F)
  VARIANT 13: note = X=Iva
  VARIANT 17: note = X=K(Ac)
  VARIANT 20: note = X=Aib

SEQ ID NO: 55 - protein, 39 aa, synthetic construct; identical to SEQ ID NO: 23
  VARIANT 2: note = X=Aib
  VARIANT 6: note = X=F(2-F)
  VARIANT 13: note = X=Iva
  VARIANT 17: note = X=K(Ac)
  VARIANT 20: note = X=Aib

SEQ ID NO: 56 - protein, 39 aa, synthetic construct
  VARIANT 2: note = X=Aib
  VARIANT 6: note = X=F(2-F)
  VARIANT 11: note = X=aMeS
YXQGTXTSDYXILLDXXAQQCFIEYLLCGGPSSGAPPPS

SEQ ID NO: 57 - protein, 39 aa, synthetic construct
  VARIANT 2: note = X=Aib
  VARIANT 6: note = X=F(2-F)
  VARIANT 13: note = X=aMeL
  VARIANT 16: note = X=aMeK
  VARIANT 17: note = X=K(Ac)
YXQGTXTSDYSIXLDXXAQQCFIEYLLCGGPSSGAPPPS

SEQ ID NO: 58 - protein, 39 aa, synthetic construct
  VARIANT 2: note = X=Aib
  VARIANT 6: note = X=F(2-F)
  VARIANT 13: note = X=aMeL
  VARIANT 16: note = X=aMeK
  VARIANT 17: note = X=K(Ac)
YXQGTXTSDYSIXLDXXAQQCXIEYLLCGGPSSGAPPPS

SEQ ID NO: 59 - protein, 39 aa, synthetic construct
  VARIANT 2: note = X=Aib
  VARIANT 6: note = X=F(2-F)
  VARIANT 13: note = X=aMeL
YXQGTXTSDYSIXLDKCAQCAFIEYLLAGGPSSGAPPPS

SEQ ID NO: 60 - protein, 39 aa, synthetic construct; identical to SEQ ID NO: 59
  VARIANT 2: note = X=Aib
  VARIANT 6: note = X=F(2-F)
  VARIANT 13: note = X=Iva

SEQ ID NO: 61 - protein, 39 aa, synthetic construct
  VARIANT 2: note = X=Aib
  VARIANT 6: note = X=F(2-F)
  VARIANT 11: note = X=aMeS
  VARIANT 13: note = X=aMeL
  VARIANT 16: note = X=aMeK
  VARIANT 17: note = X=K(Ac)
YXQGTXTSDYXIXLDXXAQXCFIEYLLCGGPSSGAPPPS

SEQ ID NO: 62 - protein, 39 aa, synthetic construct
  VARIANT 2: note = X=Aib
  VARIANT 6: note = X=F(2-F)
  VARIANT 11: note = X=aMeS
  VARIANT 13: note = X=aMeL
  VARIANT 16: note = X=aMeK
YXQGTXTSDYXIXLDXCAQCAFIEYLLAGGPSSGAPPPS

SEQ ID NO: 63 - protein, 39 aa, synthetic construct
  VARIANT 2: note = X=Aib
  VARIANT 6: note = X=F(2-F)
  VARIANT 16: note = X=K(Ac)
  VARIANT 20: note = X=Aib
HXHGTXTSDYSIYLEXKYAXCFVQWLLCGGPSSGAPPPS

SEQ ID NO: 64 - protein, 39 aa, synthetic construct
  VARIANT 2: note = X=Aib
  VARIANT 6: note = X=F(2-F)
  VARIANT 14: note = X=K(Ac)
  VARIANT 20: note = X=Aib
HXHGTXTSDYSIQXEEIAQXCFIEWLLCGGPSSGAPPPS

SEQ ID NO: 65 - protein, 39 aa, synthetic construct
  VARIANT 2: note = X=Aib
  VARIANT 6: note = X=F(2-F)
  VARIANT 14: note = X=K(Ac)
  VARIANT 20: note = X=Aib
HXHGTXTSDYSIYXEERAQXCFIEWLLCGGPSSGAPPPS

SEQ ID NO: 66 - protein, 39 aa, synthetic construct
  VARIANT 2: note = X=Aib
  VARIANT 6: note = X=F(2-F)
  VARIANT 13: note = X=Iva
  VARIANT 17: note = X=K(Ac)
  VARIANT 20: note = X=Aib
HXHGTXTSDYSIXLDKXAQXCFIEYLLCGGPSSGAPPPS

SEQ ID NO: 67 - protein, 39 aa, synthetic construct
  VARIANT 2: note = X=Aib
  VARIANT 6: note = X=F(2-F)
  VARIANT 13: note = X=aMeL
YXQGTXTSDYSIXLDKCAHCAFIEYLLAGGPSSGAPPPS

SEQ ID NO: 68 - protein, 39 aa, synthetic construct
  VARIANT 2: note = X=Aib
  VARIANT 6: note = X=F(2-F)
  VARIANT 13: note = X=aMeL
  VARIANT 19: note = X=K(Ac)
YXQGTXTSDYSIXLDKCAXCAFIEYLLAGGPSSGAPPPS

SEQ ID NO: 69 - protein, 39 aa, synthetic construct; identical to SEQ ID NO: 59
  VARIANT 2: note = X=Aib
  VARIANT 6: note = X=F(2-F)
  VARIANT 13: note = X=aMeL

SEQ ID NO: 70 - protein, 39 aa, synthetic construct
  VARIANT 2: note = X=Aib
  VARIANT 6: note = X=F(2-F)
  VARIANT 13: note = X=aMeL
HXHGTXTSDYSIXLDKCAQCAFIEYLLAGGPSSGAPPPS

SEQ ID NO: 71 - protein, 39 aa, synthetic construct; identical to SEQ ID NO: 59
  VARIANT 2: note = X=s
  VARIANT 6: note = X=F(2-F)
  VARIANT 13: note = X=aMeL

SEQ ID NO: 72 - protein, 39 aa, synthetic construct
  VARIANT 2: note = X=Aib
YXQGTFTSDYSILLDKQAQQCFIEYLLCGGPSSGAPPPS

SEQ ID NO: 73 - protein, 39 aa, synthetic construct
  VARIANT 2: note = X=Ac4c
  VARIANT 6: note = X=F(2-F)
YXQGTXTSDYSILLDKCAQCAFIEYLLEGGPSSGAPPPS

SEQ ID NO: 74 - protein, 39 aa, synthetic construct
  VARIANT 2: note = X=Ac4c
  VARIANT 6: note = X=F(2-F)
  VARIANT 17: note = X=K(Ac)
  VARIANT 20: note = X=Aib
YXQGTXTSDYSILLDKXAQXCFIEYLLCGGPSSGAPPPS

SEQ ID NO: 75 - protein, 39 aa, synthetic construct
  VARIANT 2: note = X=Ac4c
  VARIANT 6: note = X=F(2-F)
  VARIANT 20: note = X=Aib
HXHGTXTSDYSIQLEEIAQXCFIEYLLCGGPSSGAPPPS

SEQ ID NO: 76 - protein, 39 aa, synthetic construct
  VARIANT 2: note = X=Aib
  VARIANT 17: note = X=K(Ac)
  VARIANT 20: note = X=Aib
  VARIANT 21: note = X=c
  VARIANT 28: note = X=c
YXQGTFTSDYSILLDKXAQXXFIEYLLXGGPSSGAPPPS

SEQ ID NO: 77 - protein, 39 aa, synthetic construct; identical to SEQ ID NO: 76
  VARIANT 2: note = X=Aib
  VARIANT 17: note = X=K(Ac)
  VARIANT 20: note = X=Aib
  VARIANT 21: note = X=Hoc
  VARIANT 28: note = X=Hoc

SEQ ID NO: 78 - protein, 39 aa, synthetic construct; identical to SEQ ID NO: 76
  VARIANT 2: note = X=Aib
  VARIANT 17: note = X=K(Ac)
  VARIANT 20: note = X=Aib
  VARIANT 21: note = X=aMeC
  VARIANT 28: note = X=aMeC

SEQ ID NO: 79 - protein, 39 aa, synthetic construct
  VARIANT 2: note = X=Aib
  VARIANT 6: note = X=F(2-F)
  VARIANT 17: note = X=K(Ac)
  VARIANT 20: note = X=Aib
YXQGTXTSDYSIQLDKXAQXCFIEYLLCGGPSSGAPPPS

SEQ ID NO: 80 - protein, 39 aa, synthetic construct; identical to SEQ ID NO: 23
  VARIANT 2: note = X=Aib
  VARIANT 6: note = X=F(2-F)
  VARIANT 13: note = X=aMeL
  VARIANT 17: note = X=K(Ac)
  VARIANT 20: note = X=Aib

SEQ ID NO: 81 - protein, 39 aa, synthetic construct; identical to SEQ ID NO: 23
  VARIANT 2: note = X=Aib
  VARIANT 6: note = X=F(2-F)
  VARIANT 13: note = X=aMeL
  VARIANT 17: note = X=K(Ac)
  VARIANT 20: note = X=Aib

SEQ ID NO: 82 - protein, 39 aa, synthetic construct; identical to SEQ ID NO: 23
  VARIANT 2: note = X=Aib
  VARIANT 6: note = X=F(2-F)
  VARIANT 13: note = X=aMeL
  VARIANT 17: note = X=K(Ac)
  VARIANT 20: note = X=Aib

SEQ ID NO: 83 - protein, 39 aa, synthetic construct; identical to SEQ ID NO: 23
  VARIANT 2: note = X=Aib
  VARIANT 6: note = X=F(2-F)
  VARIANT 13: note = X=aMeL
  VARIANT 17: note = X=K(Ac)
  VARIANT 20: note = X=Aib

SEQ ID NO: 84 - protein, 39 aa, synthetic construct
  VARIANT 2: note = X=Aib
  VARIANT 6: note = X=F(2-F)
  VARIANT 13: note = X=aMeL
  VARIANT 16: note = X=aMeK
  VARIANT 17: note = X=K(Ac)
  VARIANT 20: note = X=Aib
YXQGTXTSDYSIXLDXXAQXKFIEYLLKGGPSSGAPPPS

SEQ ID NO: 85 - protein, 39 aa, synthetic construct
  VARIANT 2: note = X=Aib
  VARIANT 6: note = X=F(2-F)
  VARIANT 13: note = X=aMeL
  VARIANT 17: note = X=K(Ac)
  VARIANT 20: note = X=Aib
YXQGTXTSDYSIXLDKXAQXKFIEYLLKGGPSSGAPPPS

SEQ ID NO: 86 - protein, 39 aa, synthetic construct; identical to SEQ ID NO: 76
  VARIANT 2: note = X=Aib
  VARIANT 17: note = X=K(Ac)
  VARIANT 20: note = X=Aib
  VARIANT 21: note = X=Orn
  VARIANT 28: note = X=Orn

SEQ ID NO: 87 - protein, 39 aa, synthetic construct
  VARIANT 2: note = X=Aib
  VARIANT 6: note = X=F(2-F)
  VARIANT 13: note = X=aMeL
YXQGTXTSDYSIXLDKKAQKAFIEYLLAGGPSSGAPPPS

SEQ ID NO: 88 - protein, 39 aa, synthetic construct
  VARIANT 2: note = X=Aib
  VARIANT 6: note = X=F(2-F)
YXQGTXTSDYSIQLDKKAQKAFIEYLLAGGPSSGAPPPS

SEQ ID NO: 89 - protein, 39 aa, synthetic construct
YXQGTFTSDYSILLDKKAQKAFIEYLLAGGPSSGAPPPS

SEQ ID NO: 90 - protein, 39 aa, synthetic construct; identical to SEQ ID NO: 87
  VARIANT 2: note = X=Aib
  VARIANT 6: note = X=F(2-F)
  VARIANT 13: note = X=aMeL

SEQ ID NO: 91 - protein, 39 aa, synthetic construct; identical to SEQ ID NO: 87
  VARIANT 2: note = X=Aib
  VARIANT 6: note = X=F(2-F)
  VARIANT 13: note = X=aMeL

SEQ ID NO: 92 - protein, 39 aa, synthetic construct; identical to SEQ ID NO: 87
  VARIANT 2: note = X=Aib
  VARIANT 6: note = X=F(2-F)
  VARIANT 13: note = X=aMeL

SEQ ID NO: 93 - protein, 39 aa, synthetic construct; identical to SEQ ID NO: 87
  VARIANT 2: note = X=Aib
  VARIANT 6: note = X=F(2-F)
  VARIANT 13: note = X=aMeL

SEQ ID NO: 94 - protein, 39 aa, synthetic construct; identical to SEQ ID NO: 87
  VARIANT 2: note = X=Aib
  VARIANT 6: note = X=F(2-F)
  VARIANT 13: note = X=aMeL